European Patent Application EP 4 144 761 A1, published March 8, 2023. Title: Recombinant protein fused with interferon-beta mutein and antibody, and pharmaceutical composition comprising the same. Applicant: GenoPharm Inc. ABION Inc. The sequence listing filed with the application follows.

SEQUENCE LISTING (11 sequences)

SEQ ID NO: 1 - protein, 166 aa, Artificial Sequence
  Amino acid sequence of interferon beta mutein
MSYNLLGFLQRSSNFQSQKLLWQLNGTLEYCLKDRMNFDIPEEIKQLQQFQKEDAALTIYEMLQNIFAIFRQDSSSTGWNETIVENLLANVYHQINHLKTVLEEKLEKEDFTRGKLMSSLHLKRYYGRILHYLKAKEYSHCAWTIVRVEILRNFYFINRLTGYLRN

SEQ ID NO: 2 - DNA, 501 bp, Artificial Sequence
  Polynucleotide sequence of interferon beta mutein
atgtcctacaacctgctgggcttcctgcagcggtcctccaacttccagagccagaaactgctgtggcagctgaatggcaccctggaatactgcctgaaggaccggatgaacttcgacatccccgaggaaatcaagcagctgcagcagttccagaaagaggacgccgctctgaccatctacgagatgctgcagaacatcttcgccatcttccggcaggactcctcctccaccggctggaacgagacaatcgtggaaaatctgctggccaacgtgtaccaccagatcaaccacctgaaaaccgtgctggaagagaagctggaaaaagaggacttcacccggggcaagctgatgtcctccctgcacctgaagcggtactacggccggatcctgcactacctgaaggccaaagaatactcccactgcgcctggaccatcgtgcgggtggaaatcctgcggaacttctactttatcaaccggctgaccggctacctgaggaactga

SEQ ID NO: 3 - protein, 450 aa, Artificial Sequence
  Amino acid sequence of Trastuzumab heavy chain
EVQLVESGGGLVQPGGSLRLSCAASGFNIKDTYIHWVRQAPGKGLEWVARIYPTNGYTRYADSVKGRFTISADTSKNTAYLQMNSLRAEDTAVYYCSRWGGDGFYAMDYWGQGTLVTVSSASTKGPSVFPLAPSSKSTSGGTAALGCLVKDYFPEPVTVSWNSGALTSGVHTFPAVLQSSGLYSLSSVVTVPSSSLGTQTYICNVNHKPSNTKVDKKVEPKSCDKTHTCPPCPAPELLGGPSVFLFPPKPKDTLMISRTPEVTCVVVDVSHEDPEVKFNWYVDGVEVHNAKTKPREEQYNSTYRVVSVLTVLHQDWLNGKEYKCKVSNKALPAPIEKTISKAKGQPREPQVYTLPPSREEMTKNQVSLTCLVKGFYPSDIAVEWESNGQPENNYKTTPPVLDSDGSFFLYSKLTVDKSRWQQGNVFSCSVMHEALHNHYTQKSLSLSPGK

SEQ ID NO: 4 - protein, 214 aa, Artificial Sequence
  Amino acid sequence of Trastuzumab light chain
DIQMTQSPSSLSASVGDRVTITCRASQDVNTAVAWYQQKPGKAPKLLIYSASFLYSGVPSRFSGSRSGTDFTLTISSLQPEDFATYYCQQHYTTPPTFGQGTKVEIKRTVAAPSVFIFPPSDEQLKSGTASVVCLLNNFYPREAKVQWKVDNALQSGNSQESVTEQDSKDSTYSLSSTLTLSKADYEKHKVYACEVTHQGLSSPVTKSFNRGEC

SEQ ID NO: 5 - protein, 449 aa, Artificial Sequence
  Amino acid sequence of Cetuximab heavy chain
QVQLKQSGPGLVQPSQSLSITCTVSGFSLTNYGVHWVRQSPGKGLEWLGVIWSGGNTDYNTPFTSRLSINKDNSKSQVFFKMNSLQSNDTAIYYCARALTYYDYEFAYWGQGTLVTVSAASTKGPSVFPLAPSSKSTSGGTAALGCLVKDYFPEPVTVSWNSGALTSGVHTFPAVLQSSGLYSLSSVVTVPSSSLGTQTYICNVNHKPSNTKVDKKVEPKSCDKTHTCPPCPAPELLGGPSVFLFPPKPKDTLMISRTPEVTCVVVDVSHEDPEVKFNWYVDGVEVHNAKTKPREEQYNSTYRVVSVLTVLHQDWLNGKEYKCKVSNKALPAPIEKTISKAKGQPREPQVYTLPPSRDELTKNQVSLTCLVKGFYPSDIAVEWESNGQPENNYKTTPPVLDSDGSFFLYSKLTVDKSRWQQGNVFSCSVMHEALHNHYTQKSLSLSPGK

SEQ ID NO: 6 - protein, 214 aa, Artificial Sequence
  Amino acid sequence of Cetuximab light chain
DILLTQSPVILSVSPGERVSFSCRASQSIGTNIHWYQQRTNGSPRLLIKYASESISGIPSRFSGSGSGTDFTLSINSVESEDIADYYCQQNNNWPTTFGAGTKLELKRTVAAPSVFIFPPSDEQLKSGTASVVCLLNNFYPREAKVQWKVDNALQSGNSQESVTEQDSKDSTYSLSSTLTLSKADYEKHKVYACEVTHQGLSSPVTKSFNRGEC

SEQ ID NO: 7 - protein, 448 aa, Artificial Sequence
  Amino acid sequence of Atezolizumab heavy chain
EVQLVESGGGLVQPGGSLRLSCAASGFTFSDSWIHWVRQAPGKGLEWVAWISPYGGSTYYADSVKGRFTISADTSKNTAYLQMNSLRAEDTAVYYCARRHWPGGFDYWGQGTLVTVSSASTKGPSVFPLAPSSKSTSGGTAALGCLVKDYFPEPVTVSWNSGALTSGVHTFPAVLQSSGLYSLSSVVTVPSSSLGTQTYICNVNHKPSNTKVDKKVEPKSCDKTHTCPPCPAPELLGGPSVFLFPPKPKDTLMISRTPEVTCVVVDVSHEDPEVKFNWYVDGVEVHNAKTKPREEQYASTYRVVSVLTVLHQDWLNGKEYKCKVSNKALPAPIEKTISKAKGQPREPQVYTLPPSREEMTKNQVSLTCLVKGFYPSDIAVEWESNGQPENNYKTTPPVLDSDGSFFLYSKLTVDKSRWQQGNVFSCSVMHEALHNHYTQKSLSLSPGK

SEQ ID NO: 8 - protein, 214 aa, Artificial Sequence
  Amino acid sequence of Atezolizumab light chain
DIQMTQSPSSLSASVGDRVTITCRASQDVSTAVAWYQQKPGKAPKLLIYSASFLYSGVPSRFSGSGSGTDFTLTISSLQPEDFATYYCQQYLYHPATFGQGTKVEIKRTVAAPSVFIFPPSDEQLKSGTASVVCLLNNFYPREAKVQWKVDNALQSGNSQESVTEQDSKDSTYSLSSTLTLSKADYEKHKVYACEVTHQGLSSPVTKSFNRGEC

SEQ ID NO: 9 - DNA, 1896 bp, Artificial Sequence
  Polynucleotide sequence of Trastuzumab-interferon beta mutein heavy chain
gaggtgcagctggtggaatctggcggaggactggtgcagcctggcggctctctgagactgtcttgtgccgcctccggcttcaacatcaaggacacctacatccactgggtgcgacaggcccctggcaagggactggaatgggtggcccggatctatcccaccaacggctacaccagatacgccgactctgtgaagggccggttcaccatctccgccgacacctccaagaacaccgcctacctgcagatgaactccctgcgggccgaggacaccgccgtgtactactgctctagatggggaggcgacggcttctacgccatggactattggggccagggcaccctcgtgaccgtgtcctctgcttctaccaagggcccctccgtgttccctctggccccttccagcaagtctacctctggcggcacagccgctctgggctgcctcgtgaaggactacttccccgagcccgtgacagtgtcttggaactctggcgccctgacctccggcgtgcacacctttccagctgtgctgcagtccagcggcctgtactccctgtcctccgtcgtgactgtgccctccagctctctgggcacccagacctacatctgcaacgtgaaccacaagccctccaacaccaaggtggacaagaaggtggaacccaagtcctgcgacaagacccacacctgtcccccttgtcctgcccctgaactgctgggcggacccagcgtgttcctgttccccccaaagcctaaggacaccctgatgatctcccggacccccgaagtgacctgcgtggtggtggatgtgtcccacgaggaccctgaagtgaagttcaattggtacgtggacggcgtggaagtgcacaacgccaagaccaagcctagagaggaacagtacaactccacctaccgggtggtgtccgtgctgaccgtgctgcatcaggactggctgaacggcaaagagtacaagtgcaaggtgtccaacaaggccctgcctgcccccatcgaaaagaccatctccaaggccaagggccagccccgggaaccccaggtgtacacactgccccctagccgggaagagatgaccaagaaccaggtgtccctgacctgtctcgtgaaaggcttctacccctccgatatcgccgtggaatgggagtccaacggccagcctgagaacaactacaagaccaccccccctgtgctggactccgacggctcattcttcctgtacagcaagctgacagtggacaagtcccggtggcagcagggcaacgtgttctcctgctccgtgatgcacgaggccctgcacaaccactacacccagaagtccctgtccctgtctcccggaaaaggcggaggcggatctggcggcggtggttcaggcggtggatccggcatgtcctacaacctgctgggcttcctgcagcggtcctccaacttccagtcccagaaactgctgtggcagctgaatggcaccctggaatactgcctgaaggaccggatgaacttcgacatccccgaggaaatcaagcagctgcagcagttccagaaagaggacgccgctctgaccatctacgagatgctgcagaacatcttcgccatcttccggcaggactcctcctccaccggctggaacgagacaatcgtggaaaatctgctggccaacgtgtaccaccagatcaaccacctgaaaaccgtgctggaagagaagctggaaaaagaggacttcacccggggcaagctgatgtcctccctgcacctgaagcggtactacggccggatcctgcactacctgaaggccaaagaatactcccactgcgcctggaccatcgtgcgggtggaaatcctgcggaacttctactttatcaaccggctgaccggctacctgaggaactga

SEQ ID NO: 10 - DNA, 1893 bp, Artificial Sequence
  Polynucleotide sequence of Cetuximab-interferon beta mutein heavy chain
caggtgcagctgaagcagtctggccctggactggtgcagccttcccagtccctgtccatcacctgtaccgtgtccggcttctccctgaccaactacggcgtgcactgggtgcgacagtctccaggcaagggcctggaatggctgggagtgatttggagcggcggcaacaccgactacaacacccctttcacctcccggctgagcatcaacaaggacaactccaagtcccaggtgttcttcaagatgaactccctgcagtccaacgacaccgccatctactactgcgccagagccctgacctactatgactacgagttcgcctactggggccagggcaccctcgtgacagtgtctgccgcttctaccaagggcccctccgtgtttcctctggccccttccagcaagtccacctctggcggaacagccgctctgggctgcctcgtgaaggactacttccccgagcccgtgaccgtgtcctggaattctggcgctctgaccagcggagtgcacaccttccctgctgtgctgcagtcctccggcctgtactccctgtcctccgtcgtgactgtgccctccagctctctgggcacccagacctacatctgcaacgtgaaccacaagccctccaacaccaaggtggacaagaaggtggaacccaagtcctgcgacaagacccacacctgtcccccttgtcctgcccctgaactgctgggcggaccttccgtgttcctgttccccccaaagcccaaggacaccctgatgatctcccggacccccgaagtgacctgcgtggtggtggatgtgtcccacgaggaccctgaagtgaagttcaattggtacgtggacggcgtggaagtgcacaacgccaagaccaagcctagagaggaacagtacaactccacctaccgggtggtgtccgtgctgaccgtgctgcatcaggactggctgaacggcaaagagtacaagtgcaaggtgtccaacaaggccctgcctgcccccatcgaaaagaccatctccaaggccaagggacagccccgcgagccccaggtgtacacactgcctccatctcgggacgagctgaccaagaaccaggtgtccctgacctgtctcgtgaaaggcttctacccctccgacattgccgtggaatgggagtccaacggccagcccgagaacaactacaagaccaccccccctgtgctggactccgacggctcattcttcctgtacagcaagctgacagtggacaagtcccggtggcagcagggcaacgtgttctcctgctccgtgatgcacgaggccctgcacaaccactacacccagaagtccctgagcctgagccctggaaaaggcggcggaggatctggcggaggcggttctggtggcggctctggcatgtcctacaacctgctgggcttcctgcagcggtcctccaacttccagagccagaaactgctgtggcagctgaatggcaccctggaatactgcctgaaggaccggatgaacttcgacatccccgaggaaatcaagcagctgcagcagttccagaaagaggacgccgccctgacaatctacgagatgctgcagaacatcttcgccatcttccggcaggactcctcctccaccggctggaacgagacaatcgtggaaaatctgctggccaacgtgtaccaccagatcaaccacctgaaaaccgtgctggaagagaagctggaaaaagaggacttcacccggggcaagctgatgtcctccctgcacctgaagcggtactacggccggatcctgcactacctgaaggccaaagaatactcccactgcgcctggaccatcgtgcgggtggaaatcctgcggaacttctactttatcaaccggctgaccggctacctgaggaactga

SEQ ID NO: 11 - DNA, 1890 bp, Artificial Sequence
  Polynucleotide sequence of Atezolizumab-interferon beta mutein heavy chain
gaggtgcagctggttgaatctggcggaggattggttcagcctggcggctctctgagactgtcttgtgccgcttccggctttaccttctccgactcctggatccactgggtccgacaggcacctggcaaaggactggaatgggtcgcctggatctctccttacggcggctctacctactacgccgactctgtgaagggcagattcaccatctccgccgacacctccaagaacaccgcctacctgcagatgaactccctgagagccgaggacaccgccgtgtactactgtgctagaaggcattggccaggcggcttcgattattggggccagggaacactggtcaccgtgtcctctgcttccaccaagggaccctctgtgttccctctggctccttccagcaagtctacctctggcggaacagctgctctgggctgcctggtcaaggactactttcctgagcctgtgaccgtgtcttggaactctggcgctctgacatccggcgtgcacacctttccagctgtgctgcaatccagcggcctgtactctctgtcctccgtcgtgaccgtgccttcttctagcctgggcacccagacctacatctgcaatgtgaaccacaagccttccaacaccaaggtggacaagaaggtggaacccaagtcctgcgacaagacccacacctgtcctccatgtcctgctccagaactgctcggcggaccttccgtgttcctgtttcctccaaagcctaaggacaccctgatgatctctcggacccctgaagtgacctgcgtggtggtggatgtgtctcacgaggatcccgaagtgaagttcaattggtacgtggacggcgtggaagtgcacaacgccaagaccaagcctagagaggaacagtacgcctccacctacagagtggtgtccgtgctgacagtgctgcaccaggattggctgaacggcaaagagtacaagtgcaaggtgtccaacaaggccctgcctgctcctatcgaaaagaccatctccaaggccaagggccagcctcgagaaccccaggtttacaccctgcctccaagccgggaagagatgaccaagaaccaggtgtccctgacctgcctcgtgaagggcttctacccttccgacattgccgtggaatgggagagcaatggccagccagagaacaactacaagacaacccctcctgtgctggactccgacggctcattcttcctgtactccaagctgaccgtggacaagtccagatggcagcagggcaacgtgttctcctgctccgtgatgcacgaggccctgcacaatcactacacccagaagtccctgtctctgagcccaggcaaaggcggaggtggtagcggcggaggcggaagtggcggtggatctggcatgtcttacaacctgctgggcttcctgcagcggtcctccaacttccagagccagaaactgctgtggcagctgaatggcaccctggaatactgcctgaaggaccggatgaacttcgacatccccgaggaaatcaagcagctgcagcagttccagaaagaggacgccgctctgaccatctacgagatgctgcagaacatcttcgccatcttccggcaggactcctcctctaccggctggaacgagacaatcgtggaaaatctgctggccaacgtgtaccaccagatcaaccacctgaaaaccgtgctggaagagaagctggaaaaagaggacttcacccggggcaagctgatgtcctctctgcacctgaagcggtactacggccggatcctgcactacctgaaggccaaagaatactcccactgcgcctggaccatcgtgcgcgtggaaatcctgcggaacttctacttcatcaaccggctgaccggctacctgagaaactga